European Patent Specification EP 3 658 179 B1, published September 17, 2025. Title: Methods and Compositions for Heterologous repRNA Immunizations. Applicant: Janssen Vaccines & Prevention B.V. Massachusetts Institute of Technology. The sequence listing filed with the application follows.

SEQUENCE LISTING (3 sequences)

SEQ ID NO: 1 - protein, 574 aa, Artificial Sequence
  RSV-F protein, strain RSV-A2
MELLILKANAITTILTAVTFCFASGQNITEEFYQSTCSAVSKGYLSALRTGWYTSVITIELSNIKKNKCNGTDAKIKLIKQELDKYKNAVTELQLLMQSTPATNNRARRELPRFMNYTLNNAKKTNVTLSKKRKRRFLGFLLGVGSAIASGVAVSKVLHLEGEVNKIKSALLSTNKAVVSLSNGVSVLTSKVLDLKNYIDKQLLPIVNKQSCSISNIETVIEFQQKNNRLLEITREFSVNAGVTTPVSTYMLTNSELLSLINDMPITNDQKKLMSNNVQIVRQQSYSIMSIIKEEVLAYVVQLPLYGVIDTPCWKLHTSPLCTTNTKEGSNICLTRTDRGWYCDNAGSVSFFPQAETCKVQSNRVFCDTMNSLTLPSEVNLCNVDIFNPKYDCKIMTSKTDVSSSVITSLGAIVSCYGKTKCTASNKNRGIIKTFSNGCDYVSNKGVDTVSVGNTLYYVNKQEGKSLYVKGEPIINFYDPLVFPSDEFDASISQVNEKINQSLAFIRKSDELLHNVNAVKSTTNIMITTIIIVIIVILLSLIAVGLLLYCKARSTPVTLSKDQLSGINNIAFSN

SEQ ID NO: 2 - protein, 574 aa, Artificial Sequence
  RSV-preF
MELLILKANAITTILTAVTFCFASGQNITEEFYQSTCSAVSKGYLGALRTGWYTSVITIELSNIKEIKCNGTDAKVKLIKQELDKYKNAVTELQLLMQSTPATNNRARRELPRFMNYTLNNAKKTNVTLSKKRKRRFLGFLLGVGSAIASGVAVSKVLHLEGEVNKIKSALLSTNKAVVSLSNGVSVLTSKVLDLKNYIDKQLLPIVNKQSCSIPNIETVIEFQQKNNRLLEITREFSVNAGVTTPVSTYMLTNSELLSLINDMPITNDQKKLMSNNVQIVRQQSYSIMSIIKEEVLAYVVQLPLYGVIDTPCWKLHTSPLCTTNTKEGSNICLTRTDRGWYCDNAGSVSFFPQAETCKVQSNRVFCDTMNSLTLPSEVNLCNVDIFNPKYDCKIMTSKTDVSSSVITSLGAIVSCYGKTKCTASNKNRGIIKTFSNGCDYVSNKGVDTVSVGNTLYYVNKQEGKSLYVKGEPIINFYDPLVFPSDEFDASISQVNEKINQSLAFIRKSDELLHNVNAVKSTTNIMITTIIIVIIVILLSLIAVGLLLYCKARSTPVTLSKDQLSGINNIAFSN

SEQ ID NO: 3 - DNA, 9676 bp, Artificial Sequence
  repRNA construct containing the RSV preF antigen
taatacgactcactatagatgggcggcgcatgagagaagcccagaccaattacctacccaaaatggagaaagttcacgttgacatcgaggaagacagcccattcctcagagctttgcagcggagcttcccgcagtttgaggtagaagccaagcaggtcactgataatgaccatgctaatgccagagcgttttcgcatctggcttcaaaactgatcgaaacggaggtggacccatccgacacgatccttgacattggaagtgcgcccgcccgcagaatgtattctaagcacaagtatcattgtatctgtccgatgagatgtgcggaagatccggacagattgtataagtatgcaactaagctgaagaaaaactgtaaggaaataactgataaggaattggacaagaaaatgaaggagctcgccgccgtcatgagcgaccctgacctggaaactgagactatgtgcctccacgacgacgagtcgtgtcgctacgaagggcaagtcgctgtttaccaggatgtatacgcggttgacggaccgacaagtctctatcaccaagccaataagggagttagagtcgcctactggataggctttgacaccaccccttttatgtttaagaacttggctggagcatatccatcatactctaccaactgggccgacgaaaccgtgttaacggctcgtaacataggcctatgcagctctgacgttatggagcggtcacgtagagggatgtccattcttagaaagaagtatttgaaaccatccaacaatgttctattctctgttggctcgaccatctaccacgagaagagggacttactgaggagctggcacctgccgtctgtatttcacttacgtggcaagcaaaattacacatgtcggtgtgagactatagttagttgcgacgggtacgtcgttaaaagaatagctatcagtccaggcctgtatgggaagccttcaggctatgctgctacgatgcaccgcgagggattcttgtgctgcaaagtgacagacacattgaacggggagagggtctcttttcccgtgtgcacgtatgtgccagctacattgtgtgaccaaatgactggcatactggcaacagatgtcagtgcggacgacgcgcaaaaactgctggttgggctcaaccagcgtatagtcgtcaacggtcgcacccagagaaacaccaataccatgaaaaattaccttttgcccgtagtggcccaggcatttgctaggtgggcaaaggaatataaggaagatcaagaagatgaaaggccactaggactacgagatagacagttagtcatggggtgttgttgggcttttagaaggcacaagataacatctatttataagcgcccggatacccaaaccatcatcaaagtgaacagcgatttccactcattcgtgctgcccaggataggcagtaacacattggagatcgggctgagaacaagaatcaggaaaatgttagaggagcacaaggagccgtcacctctcattaccgccgaggacgtacaagaagctaagtgcgcagccgatgaggctaaggaggtgcgtgaagccgaggagttgcgcgcagctctaccacctttggcagctgatgttgaggagcccactctggaagccgatgtcgacttgatgttacaagaggctggggccggctcagtggagacacctcgtggcttgataaaggttaccagctacgatggcgaggacaagatcggctcttacgctgtgctttctccgcaggctgtactcaagagtgaaaaattatcttgcatccaccctctcgctgaacaagtcatagtgataacacactctggccgaaaagggcgttatgccgtggaaccataccatggtaaagtagtggtgccagagggacatgcaatacccgtccaggactttcaagctctgagtgaaagtgccaccattgtgtacaacgaacgtgagttcgtaaacaggtacctgcaccatattgccacacatggaggagcgctgaacactgatgaagaatattacaaaactgtcaagcccagcgagcacgacggcgaatacctgtacgacatcgacaggaaacagtgcgtcaagaaagaactagtcactgggctagggctcacaggcgagctggtggatcctcccttccatgaattcgcctacgagagtctgagaacacgaccagccgctccttaccaagtaccaaccataggggtgtatggcgtgccaggatcaggcaagtctggcatcattaaaagcgcagtcaccaaaaaagatctagtggtgagcgccaagaaagaaaactgtgcagaaattataagggacgtcaagaaaatgaaagggctggacgtcaatgccagaactgtggactcagtgctcttgaatggatgcaaacaccccgtagagaccctgtatattgacgaagcttttgcttgtcatgcaggtactctcagagcgctcatagccattataagacctaaaaaggcagtgctctgcggggatcccaaacagtgcggtttttttaacatgatgtgcctgaaagtgcattttaaccacgagatttgcacacaagtcttccacaaaagcatctctcgccgttgcactaaatctgtgacttcggtcgtctcaaccttgttttacgacaaaaaaatgagaacgacgaatccgaaagagactaagattgtgattgacactaccggcagtaccaaacctaagcaggacgatctcattctcacttgtttcagagggtgggtgaagcagttgcaaatagattacaaaggcaacgaaataatgacggcagctgcctctcaagggctgacccgtaaaggtgtgtatgccgttcggtacaaggtgaatgaaaatcctctgtacgcacccacctcagaacatgtgaacgtcctactgacccgcacggaggaccgcatcgtgtggaaaacactagccggcgacccatggataaaaacactgactgccaagtaccctgggaatttcactgccacgatagaggagtggcaagcagagcatgatgccatcatgaggcacatcttggagagaccggaccctaccgacgtcttccagaataaggcaaacgtgtgttgggccaaggctttagtgccggtgctgaagaccgctggcatagacatgaccactgaacaatggaacactgtggattattttgaaacggacaaagctcactcagcagagatagtattgaaccaactatgcgtgaggttctttggactcgatctggactccggtctattttctgcacccactgttccgttatccattaggaataatcactgggataactccccgtcgcctaacatgtacgggctgaataaagaagtggtccgtcagctctctcgcaggtacccacaactgcctcgggcagttgccactggaagagtctatgacatgaacactggtacactgcgcaattatgatccgcgcataaacctagtacctgtaaacagaagactgcctcatgctttagtcctccaccataatgaacacccacagagtgacttttcttcattcgtcagcaaattgaagggcagaactgtcctggtggtcggggaaaagttgtccgtcccaggcaaaatggttgactggttgtcagaccggcctgaggctaccttcagagctcggctggatttaggcatcccaggtgatgtgcccaaatatgacataatatttgttaatgtgaggaccccatataaataccatcactatcagcagtgtgaagaccatgccattaagcttagcatgttgaccaagaaagcttgtctgcatctgaatcccggcggaacctgtgtcagcataggttatggttacgctgacagggccagcgaaagcatcattggtgctatagcgcggctgttcaagttttcccgggtatgcaaaccgaaatcctcacttgaagagacggaagttctgtttgtattcattgggtacgatcgcaaggcccgtacgcacaatccttacaagctttcatcaaccttgaccaacatttatacaggttccagactccacgaagccggatgtgcaccctcatatcatgtggtgcgaggggatattgccacggccaccgaaggagtgattataaatgctgctaacagcaaaggacaacctggcggaggggtgtgcggagcgctgtataagaaattcccggaaagcttcgatttacagccgatcgaagtaggaaaagcgcgactggtcaaaggtgcagctaaacatatcattcatgccgtaggaccaaacttcaacaaagtttcggaggttgaaggtgacaaacagttggcagaggcttatgagtccatcgctaagattgtcaacgataacaattacaagtcagtagcgattccactgttgtccaccggcatcttttccgggaacaaagatcgactaacccaatcattgaaccatttgctgacagctttagacaccactgatgcagatgtagccatatactgcagggacaagaaatgggaaatgactctcaaggaagcagtggctaggagagaagcagtggaggagatatgcatatccgacgactcttcagtgacagaacctgatgcagagctggtgagggtgcatccgaagagttctttggctggaaggaagggctacagcacaagcgatggcaaaactttctcatatttggaagggaccaagtttcaccaggcggccaaggatatagcagaaattaatgccatgtggcccgttgcaacggaggccaatgagcaggtatgcatgtatatcctcggagaaagcatgagcagtattaggtcgaaatgccccgtcgaagagtcggaagcctccacaccacctagcacgctgccttgcttgtgcatccatgccatgactccagaaagagtacagcgcctaaaagcctcacgtccagaacaaattactgtgtgctcatcctttccattgccgaagtatagaatcactggtgtgcagaagatccaatgctcccagcctatattgttctcaccgaaagtgcctgcgtatattcatccaaggaagtatctcgtggaaacaccaccggtagacgagactccggagccatcggcagagaaccaatccacagaggggacacctgaacaaccaccacttataaccgaggatgagaccaggactagaacgcctgagccgatcatcatcgaagaggaagaagaggatagcataagtttgctgtcagatggcccgacccaccaggtgctgcaagtcgaggcagacattcacgggccgccctctgtatctagctcatcctggtccattcctcatgcatccgactttgatgtggacagtttatccatacttgacaccctggagggagctagcgtgaccagcggggcaacgtcagccgagactaactcttacttcgcaaagagtatggagtttctggcgcgaccggtgcctgcgcctcgaacagtattcaggaaccctccacatcccgctccgcgcacaagaacaccgtcacttgcacccagcagggcctgctcgagaaccagcctagtttccaccccgccaggcgtgaatagggtgatcactagagaggagctcgaggcgcttaccccgtcacgcactcctagcaggtcggtctcgagaaccagcctggtctccaacccgccaggcgtaaatagggtgattacaagagaggagtttgaggcgttcgtagcacaacaacaatgacggtttgatgcgggtgcatacatcttttcctccgacaccggtcaagggcatttacaacaaaaatcagtaaggcaaacggtgctatccgaagtggtgttggagaggaccgaattggagatttcgtatgccccgcgcctcgaccaagaaaaagaagaattactacgcaagaaattacagttaaatcccacacctgctaacagaagcagataccagtccaggaaggtggagaacatgaaagccataacagctagacgtattctgcaaggcctagggcattatttgaaggcagaaggaaaagtggagtgctaccgaaccctgcatcctgttcctttgtattcatctagtgtgaaccgtgccttttcaagccccaaggtcgcagtggaagcctgtaacgccatgttgaaagagaactttccgactgtggcttcttactgtattattccagagtacgatgcctatttggacatggttgacggagcttcatgctgcttagacactgccagtttttgccctgcaaagctgcgcagctttccaaagaaacactcctatttggaacccacaatacgatcggcagtgccttcagcgatccagaacacgctccagaacgtcctggcagctgccacaaaaagaaattgcaatgtcacgcaaatgagagaattgcccgtattggattcggcggcctttaatgtggaatgcttcaagaaatatgcgtgtaataatgaatattgggaaacgtttaaagaaaaccccatcaggcttactgaagaaaacgtggtaaattacattaccaaattaaaaggaccaaaagctgctgctctttttgcgaagacacataatttgaatatgttgcaggacataccaatggacaggtttgtaatggacttaaagagagacgtgaaagtgactccaggaacaaaacatactgaagaacggcccaaggtacaggtgatccaggctgccgatccgctagcaacagcgtatctgtgcggaatccaccgagagctggttaggagattaaatgcggtcctgcttccgaacattcatacactgtttgatatgtcggctgaagactttgacgctattatagccgagcacttccagcctggggattgtgttctggaaactgacatcgcgtcgtttgataaaagtgaggacgacgccatggctctgaccgcgttaatgattctggaagacttaggtgtggacgcagagctgttgacgctgattgaggcggctttcggcgaaatttcatcaatacatttgcccactaaaactaaatttaaattcggagccatgatgaaatctggaatgttcctcacactgtttgtgaacacagtcattaacattgtaatcgcaagcagagtgttgagagaacggctaaccggatcaccatgtgcagcattcattggagatgacaatatcgtgaaaggagtcaaatcggacaaattaatggcagacaggtgcgccacctggttgaatatggaagtcaagattatagatgctgtggtgggcgagaaagcgccttatttctgtggagggtttattttgtgtgactccgtgaccggcacagcgtgccgtgtggcagaccccctaaaaaggctgtttaagcttggcaaacctctggcagcagacgatgaacatgatgatgacaggagaagggcattgcatgaagagtcaacacgctggaaccgagtgggtattctttcagagctgtgcaaggcagtagaatcaaggtatgaaaccgtaggaacttccatcatagttatggccatgactactctagctagcagtgttaaatcattcagctacctgagaggggcccctataactctctacggctaacctgaatggactacgacatagtctagtccgccaaggccaccatggaactgctgatcctgaaggccaacgccatcaccaccatcctgaccgccgtgaccttctgcttcgccagcggccagaacatcaccgaggaattctaccagagcacctgtagcgccgtgtccaagggctacctgggcgccctgagaaccggctggtacaccagcgtgatcaccatcgagctgagcaacatcaaggaaatcaagtgcaacggcaccgacgccaaggtcaagctgatcaagcaggaactggacaagtacaagaacgccgtgaccgagctgcagctgctgatgcagagcacccccgccaccaacaaccgggccagacgcgagctgccccggttcatgaactacaccctgaacaacgccaaaaagaccaacgtgaccctgagcaagaagcggaagcggcggttcctgggcttcctgctgggcgtgggcagcgccattgcttctggcgtggccgtgtctaaggtgctgcacctggaaggcgaagtgaacaagatcaagagcgccctgctgagcaccaacaaggccgtggtgtccctgagcaacggcgtgtccgtgctgaccagcaaggtgctggatctgaagaactacatcgacaagcagctgctgcccatcgtgaacaagcagagctgcagcatccccaacatcgagacagtgatcgagttccagcagaagaacaaccggctgctggaaatcacccgcgagttcagcgtgaacgccggcgtgaccacccccgtgtccacctacatgctgaccaacagcgagctgctgagcctgatcaacgacatgcccatcaccaacgaccagaaaaagctgatgagcaacaacgtgcagatcgtgcggcagcagagctactccatcatgagcatcatcaaagaagaggtgctggcctacgtggtgcagctgcccctgtacggcgtgatcgacaccccctgctggaagctgcacaccagccccctgtgcaccaccaacaccaaagagggcagcaacatctgcctgacccggaccgaccggggctggtactgcgataatgccggctcagtctcattctttccacaggccgagacatgcaaggtgcagagcaaccgggtgttctgcgacaccatgaacagcctgaccctgccctccgaagtgaacctgtgcaacgtggacatcttcaaccctaagtacgactgcaagatcatgacctccaagaccgacgtgtccagctccgtgatcacctccctgggcgccatcgtgtcctgctacggcaagaccaagtgcaccgccagcaacaagaaccggggcatcatcaagaccttcagcaacggctgcgactacgtgtccaacaagggggtggacaccgtgtccgtgggcaacaccctgtactacgtgaacaaacaggaaggcaagagcctgtacgtgaagggcgagcccatcatcaacttctacgaccccctggtgttccccagcgacgagttcgacgccagcatcagccaggtcaacgagaagatcaaccagagcctggccttcatcagaaagagcgacgagctgctgcacaatgtgaatgccgtgaagtccaccaccaatatcatgatcaccacaatcatcatcgtgatcatcgtcatcctgctgtccctgatcgccgtgggcctgctgctgtactgcaaggccagatccacccctgtgaccctgtccaaggaccagctgagcggcatcaacaatatcgccttctccaactaataatatgttacgtgcaaaggtgattgtcaccccccgaaagaccatattgtgacacaccctcagtatcacgcccaaacatttacagccgcggtgtcaaaaaccgcgtggacgtggttaacatccctgctgggaggatcagccgtaattattataattggcttggtgctggctactattgtggccatgtacgtgctgaccaaccagaaacataattgaatacagcagcaattggcaagctgcttacatagaactcgcggcgattggcatgccgccttaaaatttttattttatttttcttttcttttccgaatcggattttgtttttaatatttcaaaaaaaaaaaaaaaaaaaaaaaaaaaaaaaaa